European Patent Specification EP 3 792 360 B1, published April 1, 2026. Title: Marburg Virus Vaccine with Human Replication-Deficient Adenovirus as Vector. Applicant: Academy of Military Medical Science, PLA. The sequence listing filed with the application follows.

SEQUENCE LISTING (2 sequences)

SEQ ID NO: 1 - DNA, 2088 bp, Marburg virus
ccaagcttgccgccaccatggacgccatgaagcggggcctctgctgtgttctgctgctctgcggcgccgtgttcgtgagtaactcgttacccattctggagattgccagcaacatccagccccagaacgtggattccgtgtgctccggcaccctgcagaagaccgaagatgtccatctcatgggcttcaccctgtccgggcagaaggtcgccgactcgcccctggaggccagcaagcgctgggccttccgcgcaggcgtccctcctaagaacgtggaatacacggagggagaggaggccaagacttgttacaacatctcagtaaccgacccctccggtaaaagtctcctgctcgaccctccgacgaacatccgcgactaccccaagtgcaagacaatccaccacattcagggccagaatccgcacgcccagggtatcgccctgcacctgtggggcgcttttttcctgtacgaccgaatcgcctccaccaccatgtaccgggggaaggtttttaccgagggcaatatcgccgccatgattgtgaataagaccgtccacaagatgatcttctccaggcaggggcagggataccggcacatgaacctgacctccactaacaagtactggactagttccaacggtacccagaccaacgacactggctgctttgggaccctccaggagtacaactccaccaaaaaccagacttgtgccccgtccaaaaagcccctgcccctgcctaccgcccacccggaagtgaagctgacatctacatcgaccgacgcaacaaaactcaatactaccgaccccaatagtgacgacgaggacctgaccaccagtggcagcggctccggcgagcaggagccatacaccacctcggacgcagcaaccaagcagggcctgtcgtccacgatgccgcctaccccgtcgccccagccctcgaccccgcagcagggcggcaataataccaaccattctcagggggtcgttaccgagcccggcaagaccaacacgactgctcagccatccatgccaccccacaacaccaccactatctcgaccaacaacacttcaaagcacaacctctcgacccccagtgtcccaatccagaacgccaccaactataacacgcagtccacagcgcccgagaacgagcagacaagtgccccctctaagacgaccctcctccccaccgagaaccccacaaccgccaagtccaccaactcaaccaagtcccccacgacgaccgttcccaacaccaccaacaagtactcaacctctccttcgcctaccccaaactccaccgcgcagcaccttgtgtacttccgccggaagcgaaacatcctgtggcgcgagggagacatgttccctttcctcgatggactgatcaacgcccccatcgactttgatccagtccccaacaccaagacgatcttcgatgaaagtagtagttcgggggctagtgcagaagaggaccagcatgcgagtcctaacatctccctgaccctctcctacttccccaaggtgaacgagaataccgcccactccggcgagaatgagaacgattgcgatgccgaactgaggatctggagtgtgcaggaggacgacctggcggctggcctgtcttggatccccttctttgggccgggcatcgagggcctgtacaccgccggcctgattaaaaaccagaacaacctggtttgccgcctgagaagactggcaaaccagactgccaagtccctggaactgctcttacgcgtcaccaccgaggagcggaccttttcgctcatcaaccgccacgccatcgacttcctgctggcccggtggggcggtacgtgcaaagtgctgggccccgactgctgcatcggcatcgaggatctcagccgcaacatctctgagcaaatcgatcagatcaagaaggatgagcagaaggaaggtaccggctggggcctgggggggaagtggtggaccagtgactggggcgtgctgactaacctgggcatcctgctgctgctatcgatcgccgtgctcatcgccctgtcttgcatctgccgtatcttcaccaaatatatcggctaagtcgacgtct

SEQ ID NO: 2 - DNA, 2073 bp, Marburg virus
ccaagcttgccgccaccatgaaaaccacatgtctccttatcagtcttatcttaatccaaggggtaaaaactctccctattttagagatagccagtaacattcaaccccaaaatgtggattcagtatgctccgggactctccagaagacagaagacgttcatctgatgggattcacactgagcgggcaaaaagttgctgattcccctttagaggcatccaaacgatgggccttcagggcaggtgtacctcccaagaatgttgagtatacagaaggggaggaagctaaaacatgttacaatataagtgtaacggatccctctggaaaatccttgctgttagatcctcctaccaacatccgtgactatcctaaatgcaaaactatccatcatattcaaggtcaaaaccctcatgcacaggggatcgctctccatttgtggggagcatttttcttgtatgatcgcatcgcctccacaacgatgtatcgaggcaaagtcttcactgaagggaacatagcagctatgattgtcaataagacagtgcacaaaatgattttctcgaggcaaggacaagggtaccgtcacatgaacctaacttctactaataaatattggacaagtagcaacggaacgcaaacgaatgacactggatgcttcggtactcttcaagaatataattctacaaagaaccaaacatgtgctccgtccaaaaaacctttaccactgcccacagcccatccggaggtcaagctcactagcacctcaactgatgccaccaaactcaataccacagacccaaacagtgatgatgaggacctcacaacatctggctcagggtctggagaacaggaaccttacacaacttctgacgcagccacgaagcaagggctttcatcaacaatgccgcccactccctcaccacaaccaagcacgccacagcaaggaggaaacaacacgaaccattcccaaggtgttgtgactgaacccggcaaaaccaacacaactgcacaaccgtccatgccccctcacaacactactacaatctctactaacaacacctccaagcacaacctcagcactccctctgtaccaatacaaaatgccactaattacaacacacagagcacggcccctgaaaatgagcaaaccagtgccccctcgaaaacaaccctgcttccaacagaaaatcctacaacagcaaagagcaccaatagtacaaaaagccccactacaacagtaccaaatacgacaaataagtattccaccagtccctcccccacccccaactcgactgcacaacatcttgtatatttcagaaggaaacgaaatattctctggagggaaggcgacatgttcccttttctggatgggttaataaatgctccgattgattttgatccggttccaaatacaaagacaatctttgatgaatcctctagttctggtgcttcagctgaggaagatcagcatgcctcccctaatatcagtttaactttatcttactttcctaaggtaaatgaaaacactgcccactctggagaaaatgaaaatgattgtgatgcagagttaagaatttggagtgttcaggaggacgacctggcagcaggactcagttggataccgttttttggccctggaatcgaaggactttatactgctggtttaattaaaaatcaaaataatttggtttgcaggttgaggcgtctagccaatcagactgccaaatccttggaactcttattaagagtcacaaccgaggaaagaacattttccttaatcaatagacatgccattgattttttactcgcaaggtggggaggaacatgcaaagtgcttggacctgattgttgcatcggaatagaagacttgtccagaaatatttcagaacaaattgatcaaatcaaaaaggacgaacaaaaagaggggactggttggggtctgggtggtaaatggtggacatcagactggggtgttcttactaacttgggcatcttgctactactgtccatagctgtcttaattgctctgtcctgtatttgtcgtatttttactaaatatattggataagtcgacgtct